European Patent Application EP 4 782 542 A1, published July 29, 2026. Title: 一种基于合成细胞器的目标产物回收方法、DNA构建体和表达系统. Applicant: 小熊猫有限公司. The sequence listing filed with the application follows.

SEQUENCE LISTING (19 sequences)

SEQ ID NO: 1 - protein, 232 aa, synthetic construct
MSKGEELFTGVVPILVELDGDVNGHKFSVRGEGEGDATNGKLTLKFICTTGKLPVPWPTLVTTLTYGVQCFSRYPDHMKRHDFFKSAMPEGYVQERTISFKDDGTYKTRAEVKFEGDTLVNRIELKGIDFKEDGNILGHKLEYNFNSHNVYITADKQKNGIKANFKIRHNVEDGSVQLADHYQQNTPIGDGPVLLPDNHYLSTQSVLSKDPNEKRDHMVLLEFVTAAGITHG

SEQ ID NO: 2 - RNA, 816 nt, synthetic construct
  source 1..816: mol_type = other RNA
cagcagcagcagcagcagcagcagcagcagcagcagcagcagcagcagcagcagcagcagcagcagcagcagcagcagcagcagcagcagcagcagcagcagcagcagcagcagcagcagcagcagcagcagcagcagcagagacggagctcgtcgacgcggccgcaagcttggtaccgagctcggatcctaaggtacctaattgcctagaaaacatgaggatcacccatgtctgcaggtcgactctagaaaacatgaggatcacccatgtctgcagtattcccgggttcattagatcctaaggtacctaattgcctagaaaacatgaggatcacccatgtctgcaggtcgactctagaaaacatgaggatcacccatgtctgcagtattcccgggttcattagatcctaaggtacctaattgcctagaaaacatgaggatcacccatgtctgcaggtcgactctagaaaacatgaggatcacccatgtctgcagtattcccgggttcattagatcctaaggtacctaattgcctagaaaacatgaggatcacccatgtctgcaggtcgactctagaaaacatgaggatcacccatgtctgcagtattcccgggttcattagatcctaaggtacctaattgcctagaaaacatgaggatcacccatgtctgcaggtcgactctagaaaacatgaggatcacccatgtctgcagtattcccgggttcattagatcctaaggtacctaattgcctagaaaacatgaggatcacccatgtctgcaggtcgactctagaaaacatgaggatcacccatgt

SEQ ID NO: 3 - protein, 258 aa, synthetic construct
MASNFTQFVLVDNGGTGDVTVAPSNFANGVAEWISSNSRSQAYKVTCSVRQSSAQNRKYTIKVEVPKVATQTVGGVELPVAAWRSYLNMELTIPIFATNSDCELIVKAMQGLLKDGNPIPSAIAANSGIYANFTQFVLVDNGGTGDVTVAPSNFANGVAEWISSNSRSQAYKVTCSVRQSSAQNRKYTIKVEVPKVATQTVGGVELPVAAWRSYLNMELTIPIFATNSDCELIVKAMQGLLKDGNPIPSAIAANSGIY

SEQ ID NO: 4 - protein, 5 aa, synthetic construct
GSHHW

SEQ ID NO: 5 - protein, 487 aa, synthetic construct
MILKILNEIASIGSTKQKQAILEKNKDNELLKRVYRLTYSRGLQYYIKKWPKPGIATQSFGMLTLTDMLDFIEFTLATRKLTGNAAIEELTGYITDGKKDDVEVLRRVMMRDLECGASVSIANKVWPGLIPEQPQMLASSYDEKGINKNIKFPAFAQLKADGARCFAEVRGDELDDVRLLSRAGNEYLGLDLLKEELIKMTAEARQIHPEGVLIDGELVYHEQVKKEPEGLDFLFDAYPENSKAKEFAEVAESRTASNGIANKSLKGTISEKEAQCMKFQVWDYVPLVEIYSLPAFRLKYDVRFSKLEQMTSGYDKVILIENQVVNNLDEAKVIYKKYIDQGLEGIILKNIDGLWENARSKNLYKFKEVIDVDLKIVGIYPHRKDPTKAGGFILESECGKIKVNAGSGLKDKAGVKSHELDRTRIMENQNYYIGKILECECNGWLKSDGRTDYVKLFLPIAIRLREDKTKANTFEDVFGDFHEVTGL

SEQ ID NO: 6 - protein, 142 aa, synthetic construct
RDHMVLHEYVNAAGITGGSGGRDHMVLHEYVNAAGITGGSGGRDHMVLHEYVNAAGITGGSGGRDHMVLHEYVNAAGITGGSGGRDHMVLHEYVNAAGITGGSGGRDHMVLHEYVNAAGITGGSGGRDHMVLHEYVNAAGIT

SEQ ID NO: 7 - protein, 214 aa, synthetic construct
MSKGEELFTGVVPILVELDGDVNGHKFSVRGEGEGDATIGKLTLKFICTTGKLPVPWPTLVTTLTYGVQCFSRYPDHMKRHDFFKSAMPEGYVQERTISFKDDGKYKTRAVVKFEGDTLVNRIELKGTDFKEDGNILGHKLEYNFNSHNVYITADKQKNGIKANFTVRHNVEDGSVQLADHYQQNTPIGDGPVLLPDNHYLSTQTVLSKDPNEK

SEQ ID NO: 8 - protein, 231 aa, synthetic construct
MSELIKENMHMKLYMEGTVNNHHFKCTSEGEGKPYEGTQTMRIKAVEGGPLPFAFDILATSFMYGSKTFINHTQGIPDFFKQSFPEGFTWERVTTYEDGGVLTATQDTSLQDGCLIYNVKIRGVNFPSNGPVMQKKTLGWEASTETLYPADGGLEGRADMALKLVGGGHLICNLKTTYRSKKPAKNLKMPGVYYVDRRLERIKEADKETYVEQHEVAVARYCDLPSKLGHR

SEQ ID NO: 9 - protein, 166 aa, synthetic construct
SKGPGRGDSPYSGRGDSPYSGRGDSPYSGRGDSPYSGRGDSPYSGRGDSPYSGRGDSPYSGRGDSPYSGRGDSPYSGRGDSPYSGRGDSPYSGRGDSPYSGRGDSPYSGRGDSPYSGRGDSPYSGRGDSPYSGRGDSPYSGRGDSPYSGRGDSPYSGRGDSPYSGY

SEQ ID NO: 10 - RNA, 1450 nt, synthetic construct
  source 1..1450: mol_type = other RNA
agtttgatcatggctcagattgaacgctggcggcaggcctaacacatgcaagtcgaacggtaacaggaagcagcttgctgctttgctgacgagtggcggacgggtgagtaatgtctgggaaactgcctgatggagggggataactactggaaacggtagctaataccgcataacgtcgcaagcacaaagagggggaccttagggcctcttgccatcggatgtgcccagatgggattagctagtaggtggggtaacggctcacctaggcgacgatccctagctggtctgagaggatgaccagcaacactggaactgagacacggtccagactcctacgggaggcagcagtggggaatattgcacaatgggcgcaagcctgatgcagccatgcngcgtgtatgaagaaggccttcgggttgtaaagtactttcagcggggaggaagggagtaaagttaatacctttgctcattgacgttacccgcagaagaagcaccggctaactccgtgccagcagccgcggtaatacggagggtgcaagcgttaatcggaattactgggcgtaaagcgcacgcaggcggtttgttaagtcagatgtgaaatccccgggctcaacctgggaactgcatctgatactggcaagcttgagtctcgtagaggggggtagaattccaggtgtagcggtgaaatgcgtagagatctggaggaataccggtggcgaaggcggccccctggacgaagactgacgctcaggtgcgaaagcgtggggagcaaacaggattagataccctggtagtccacgccgtaaacgatgtcgacttggaggttgtgcccttgaggcgtggcttccgganntaacgcgttaagtcgaccgcctggggagtacggccgcaaggttaaaactcaaatgaattgacgggggccgcacaagcggtggagcatgtggtttaattcgatgcaacgcgaagaaccttacctggtcttgacatccacggaagttttcagagatgagaatgtgccttcgggaaccgtgagacaggtgctgcatggctgtcgtcagctcgtgttgtgaaatgttgggttaagtcccgcaacgagcgcaacccttatcctttgttgccagcggtccggccgggaactcaaaggagactgccagtgataaactggaggaaggtggggatgacgtcaagtcatcatggcccttacgaccagggctacacacgtgctacaatggcgcatacaaagagaagcgacctcgcgagagcaagcggacctcataaagtgcgtcgtagtccggattggagtctgcaactcgactccatgaagtcggaatcgctagtaatcgtggatcagaatgccacggtgaatacgttcccgggccttgtacacaccgcccgtcacaccatgggagtgggttgcaaaagaagtaggtagcttaacttcgggagggcg

SEQ ID NO: 11 - RNA, 28 nt, synthetic construct
  source 1..28: mol_type = other RNA
gttcactgccgtataggcagctaagaaa

SEQ ID NO: 12 - protein, 187 aa, synthetic construct
MDHYLDIRLRPDPEFPPAQLMSVLFGKLAQALVAQGGDRIGVSFPDLDESRSRLGERLRIHASADDLRALLARPWLEGLRDHLQFGEPAVVPHPTPYRQVSRVQAKSNPERLRRRLMRRHDLSEEEARKRIPDTVARALDLPFVTLRSQSTGQHFRLFIRHGPLQVTAEEGGFTCYGLSKGGFVPWF

SEQ ID NO: 13 - protein, 196 aa, synthetic construct
MGSLITLVELEWLEHQLIVQLSERLKGQIAKVGELLCECLKKGGKILICGNGGSAADAQHFAAELSGRYKKERKALAGIALTTDTSALSAIGNDYGFEFVFSRQVEALGNEKDVLIGISTSGKSPNVLEALKKAKELNMLCLGLSGKGGGMMNKLCDHNLVVPSDTARIQEMHILIIHTLCQIIDESFLEHHHHHH

SEQ ID NO: 14 - protein, 242 aa, synthetic construct
MGHHHHHHGGLALVATGNDTTTKPDLYYLKNSEAINSLALLPPPPAVGSIAFLNDQAMYEQGRLLRNTERGKLAAEDANLSSGGVANAFSGAFGSPITEKDAPALHKLLTNMIEDAGDLATRSAKDHYMRIRPFAFYGVSTCNTTEQDKLSKNGSYPSGHTSIGWATALVLAEINPQRQNEILKRGYELGQSRVICGYHWQSDVDAARVVGSAVVATLHTNPEFQAQLIKAKIEFKQHQKEL

SEQ ID NO: 15 - RNA, 622 nt, synthetic construct
  source 1..622: mol_type = other RNA
cagcagcagcagcagcagcagcagcagcagcagcagcagcagcagcagcagcagcagcagcagcagcagcagcagcagcagcagcagcagcagcagcagcagcagcagcagcagcagcagcagcagcagcagcagcagagacggagctcgtcgacgcggccaagcttggtaccgagctcgggccctgaagaagggcccctcgactaagtccaactactaaactgggccctgaagaagggcccatatagggccctgaagaagggcccctcgactaagtccaactactaaactgggccctgaagaagggcccatatagggccctgaagaagggcccctcgactaagtccaactactaaactgggccctgaagaagggcccatatagatcaagcttggtaccgagctcgggccctgaagaagggcccctcgactaagtccactactaaactgggccctgaagaagggcccatatagggccctgaagaagggcccctcgactaagtccaactactaaactgggccctgaagaagggcccatatagggccctgaagaagggcccctcgactaagtccaactactaaactgggccctgaagaagggcccatatatcgagtaaggatct

SEQ ID NO: 16 - protein, 418 aa, synthetic construct
MKHSSDICIVGAGISGLTCASHLLDSPACRGLSLRIFDMQQEAGGRIRSKMLDGKASIELGAGRYSPQLHPHFQSAMQHYSQKSEVYPFTQLKFKSHVQQKLKRAMNELSPRLKEHGKESFLQFVSRYQGHDSAVGMIRSMGYDALFLPDISAEMAYDIVGKHPEIQSVTDNDANQWFAAETGFAGLIQGIKAKVKAAGARFSLGYRLLSVRTDGDGYLLQLAGDDGWKLEHRTRHLILAIPPSAMAGLNVDFPEAWSGARYGSLPLFKGFLTYGEPWWLDYKLDDQVLIVDNPLRKIYFKGDKYLFFYTDSEMANYWRGCVAEGEDGYLEQIRTHLASALGIVRERIPQPLAHVHKYWAHGVEFCRDSDIDHPSALSHRDSGIIACSDAYTEHCGWMEGGLLSAREASRLLLQRIAA

SEQ ID NO: 17 - protein, 998 aa, synthetic construct
MSILDFPRIHFRGWARVNAPTANRDPHGHIDMASNTVAMAGEPFDLARHPTEFHRHLRSLGPRFGLDGRADPEGPFSLAEGYNAAGNNHFSWESATVSHVQWDGGEADRGDGLVGARLALWGHYNDYLRTTFNRARWVDSDPTRRDAAQIYAGQFTISPAGAGPGTPWLFTADIDDSHGARWTRGGHIAERGGHFLDEEFGLARLFQFSVPKDHPHFLFHPGPFDSEAWRRLQLALEDDDVLGLTVQYALFNMSTPPQPNSPVFHDMVGVVGLWRRGELASYPAGRLLRPRQPGLGDLTLRVNGGRVALNLACAIPFSTRAAQPSAPDRLTPDLGAKLPLGDLLLRDEDGALLARVPQALYQDYWTNHGIVDLPLLREPRGSLTLSSELAEWREQDWVTQSDASNLYLEAPDRRHGRFFPESIALRSYFRGEARARPDIPHRIEGMGLVGVESRQDGDAAEWRLTGLRPGPARIVLDDGAEAIPLRVLPDDWALDDATVEEVDYAFLYRHVMAYYELVYPFMSDKVFSLADRCKCETYARLMWQMCDPQNRNKSYYMPSTRELSAPKARLFLKYLAHVEGQARLQAPPPAGPARIESKAQLAAELRKAVDLELSVMLQYLYAAYSIPNYAQGQQRVRDGAWTAEQLQLACGSGDRRRDGGIRAALLEIAHEEMIHYLVVNNLLMALGEPFYAGVPLMGEAARQAFGLDTEFALEPFSESTLARFVRLEWPHFIPAPGKSIADCYAAIRQAFLDLPDLFGGEAGKRGGEHHLFLNELTNRAHPGYQLEVFDRDSALFGIAFVTDQGEGGALDSPHYEHSHFQRLREMSARIMAQSAPFEPALPALRNPVLDESPGCQRVADGRARALMALYQGVYELMFAMMAQHFAVKPLGSLRRSRLMNAAIDLMTGLLRPLSCALMNLPSGIAGRTAGPPLPGPVDTRSYDDYALGCRMLARRCERLLEQASMLEPGWLPDAQMELLDFYRRQMLDLACGKLSREA

SEQ ID NO: 18 - protein, 191 aa, synthetic construct
MENREPPLLPARWSSAYVSYWSPMLPDDQLTSGYCWFDYERDICRIDGLFNPWSERDTGYRLWMSEVGNAASGRTWKQKVAYGRERTALGEQLCERPLDDETGPFAELFLPRDVLRRLGARHIGRRVVLGREADGWRYQRPGKGPSTLYLDAASGTPLRMVTGDEASRASLRDFPNVSEAEIPDAVFAAKR

SEQ ID NO: 19 - protein, 428 aa, synthetic construct
KRAIIVGGGLAGGLTAIYLAKRGYEVHVVEKRGDPLRDLSSYVDVVSSRAIGVSMTVRGIKSVLAAGIPRAELDACGEPIVAMAFSVGGQYRMRELKPLEDFRPLSLNRAAFQKLLNKYANLAGVRYYFEHKCLDVDLDGKSVLIQGKDGQPQRLQGDMIIGADGAHSAVRQAMQSGLRRFEFQQTFFRHGYKTLVLPDAQALGYRKDTLYFFGMDSGGLFAGRAATIPDGSVSIAVCLPYSGSPSLTTTDEPTMRAFFDRYFGGLPRDARDEMLRQFLAKPSNDLINVRSSTFHYKGNVLLLGDAAHATAPFLGQGMNMALEDARTFVELLDRHQGDQDKAFPEFTELRKVQADAMQDMARANYDVLSCSNPIFFMRARYTRYMHSKFPGLYPPDMAEKLYFTSEPYDRLQQIQRKQNVWYKIGRVN